European Patent Application EP 4 603 580 A1, published August 20, 2025. Title: Method of fermentative vanillin or 4-vinylguaiacol production. Applicant: Phytowelt Greentechnologies GmbH. Application EP. The sequence listing filed with the application follows.

SEQUENCE LISTING (8 sequences)

SEQ ID NO: 1 - DNA, 507 bp, Enterobacter sp. Px6-4
  source 1..507: mol_type = unassigned DNA
  misc_feature 1..507: note = FADse nucleotide sequence
atgaacacatttgacaagcacgatcttagcggattcgttggtaagcacttggtatacacttacgataacgggtgggaatatgagatttatgtgaagaatgagaataccctggactaccgtatccactctggtttggttggcaaccgttgggtcaaagatcagcaagcgtatattgtgcgcgtgggcgaatctatctataagatcagctggaccgagccgacaggaacggatgtttcactgattgtgaacttaggtgactcactgtttcacggcacaatcttctttccgcgttgggtaatgaataatccagagaagactgtgtgctttcagaatgatcacattcctctgatgaatagttaccgtgatgccggtccagcgtatccgactgaggtaattgacgagttcgcaacgattacgttcgtgcgtgattgtggggcaaacaatgagtcagtcatcgcctgtgctgcttcggaactgcccaagaatttcccagataacttaaaataa

SEQ ID NO: 2 - protein, 168 aa, Enterobacter sp. Px6-4
  REGION 1..168: note = FADse amino acid sequence
MNTFDKHDLSGFVGKHLVYTYDNGWEYEIYVKNENTLDYRIHSGLVGNRWVKDQQAYIVRVGESIYKISWTEPTGTDVSLIVNLGDSLFHGTIFFPRWVMNNPEKTVCFQNDHIPLMNSYRDAGPAYPTEVIDEFATITFVRDCGANNESVIACAASELPKNFPDNLK

SEQ ID NO: 3 - DNA, 1809 bp, Myceliophthora thermophila
  source 1..1809: mol_type = unassigned DNA
  misc_feature 1..1809: gene = TtAdo nucleotide sequence
atggcacatattcatgatctcgcaccggaagtatcgaactactcctcgggcagactaacgcccccaacgcccgtgcgttttcctcgaacgcccgtcttcgcctcaatgaataagccgtgccgttttgaaggggatgtatttgacctcgaggtctccggcgcaatcccacctgacatcgacgggacgttcttccgagtccagccagatcatagattccctccgcttttcgaagatgatatccatttcaatggtgatggatctgtgaccgccattcggatctccggcggtcacgccgacttacgtcaaagatatgtacgaactgagagatatctgctggaaacgcgggcacgccgttcgctgtttgggcgttacagaaacccgtggaccgacaacgaaagtgttcggggcgtgatacgtaccgcatcaaacactaacgtggtattctggcgcggggcgctgttagcgatgaaagaagatggccctccttttgcgatggacccggtcacgttagaaacactcggtcgctacgattttgaaggacagatactctcccccacatttacggcccacccgaaaatagatcctgacaccggggagatggtctgctttgcctatgaggccggaggtgacggctcagattgtagtgtcgacgtagcggtctggaccgtcgatgccgacggtaaaaaagtggaagagtgctggtacaaggcgccctttgccgggatgatacatgactgtggaatcaccaaaaactgggtggttctaccattaacgcccataaagatggaccttgaacgcatgaagagaggcgggaataaattcgcctgggaccccagcgaagatcagtggtatggcgtagtaccccgccgtggtgccaagtctgatgatattatatggtttagagcggataatggttttcacggtcatgtcgcgggctgctatgaattaccttcgggtgagatagtttttgatctgaccgtggccgacggaaacgttttcttctttttcccgcccgacgataacattacaccgcctgcagacggcgtggccaagaggaaccggttatcatccccgacggtacgctggatatttgacccgaaggcgaaaaagtcagccattcgtactgaagcagctggcgatgctgatatctgggttgctgatgaaagggtcaaaccggcattaacgtggccgacgaacggcgaattcagccgtatcgacgacagatatgttaccaaaccatatcggcacttctggcaggccgtggttgatccaacgcgaccgtacgatttcgagaagtgtgggcctcctgctggggggctgttcaactgtctggggcattatacctggagcgatcaaaactatcatcacggtcacaacactggagaccctagcggcgacgggcgcagtaatggttcagctgaagaagccaccgccgggaagttcggtctacaggatgtttattttgcggggccaacaatgacttttcaggagccaacattcattccacggcagggtgctgcagagggggagggctatttgatagccttactcaaccatctcgatgagttacggaacgatgtagtgattttcgaagcgcgtaatctggggaaagggccgctggcggttatacatctgccgctaaagctgaagctgggacttcatggcaactgggtggactcccgcgagattgaggcatggcggagaagaagagcagaaaatggcgatgtcggcccgttacgggtggcgaaagagccgctaccctggcaaaagaaattcgccgccgcagcccaaaacggcagtaatggcgtt

SEQ ID NO: 4 - protein, 604 aa, Myceliophthora thermophila
  REGION 1..603: note = TtAdo amino acid sequence
MAHIHDLAPEVSNYSSGRLTPPTPVRFPRTPVFASMNKPCRFEGDVFDLEVSGAIPPDIDGTFFRVQPDHRFPPLFEDDIHFNGDGSVTAIRISGGHADLRQRYVRTERYLLETRARRSLFGRYRNPWTDNESVRGVIRTASNTNVVFWRGALLAMKEDGPPFAMDPVTLETLGRYDFEGQILSPTFTAHPKIDPDTGEMVCFAYEAGGDGSDCSVDVAVWTVDADGKKVEECWYKAPFAGMIHDCGITKNWVVLPLTPIKMDLERMKRGGNKFAWDPSEDQWYGVVPRRGAKSDDIIWFRADNGFHGHVAGCYELPSGEIVFDLTVADGNVFFFFPPDDNITPPADGVAKRNRLSSPTVRWIFDPKAKKSAIRTEAAGDADIWVADERVKPALTWPTNGEFSRIDDRYVTKPYRHFWQAVVDPTRPYDFEKCGPPAGGLFNCLGHYTWSDQNYHHGHNTGDPSGDGRSNGSAEEATAGKFGLQDVYFAGPTMTFQEPTFIPRQGAAEGEGYLIALLNHLDELRNDVVIFEARNLGKGPLAVIHLPLKLKLGLHGNWVDSREIEAWRRRRAENGDVGPLRVAKEPLPWQKKFAAAAQNGSNGVG

SEQ ID NO: 5 - DNA, 1788 bp, Thermothielavioides terrestris
  source 1..1788: mol_type = unassigned DNA
  misc_feature 1..1788: gene = TtAdo2 nucleotide sequence
atggcacatatccatgaacttgctgcagaaatcagtaactacgctaacaaccgactgaccgacccttcaaaagtcagatttcctcgaacgcccgtcttcgcctcaatgaataaaccttcccgttttgaaggggatgtatttgaccttgaaattagcggcactatccctgctgatattgacgggacgttcttccgagtccagccagatcatagattccctccgcttttcgaagatgatatccatttcaatggtgatggatctgtcactgctgtccggatatccggcggtcacgccgacttgaaacaaagatatgtgcacacggatcgttatgtgcacgaaacaagggcacgccgttcgctgtttgggcgttacagaaacccgtggaccgacaacgaatcggtgaagggggtgatacgtaccgcatcaaacactaacgtggtattctggcgcggcgtgttactggcgcttaaagaagatggccctccttttgcgatggacccggtcacgttagaaacactcggtcgctacgattttgaaggacagatactctcccccacatttacggcccatcctaagtttgatccagacaccggggagatggtctgctttgcctatgaggccggaggtgacggctcagattgtagtgtcgacgtagcggtctggacaatcgatagagacggaaaaaaaactgaagagtgctggtacaaggcgccctttgccgggatgatacatgactgtggaatcagcaaaaactggttagtacttgcattaactcccataaagatggaccttgaacgcatgaagagaggcgggaataaattcgcctgggacccgaacgaagatcagtggtacgctgtcgtgccgcgaaggggcggaaagtcagaggatatcacctggtttagagcggataatggttttcacggtcatgtcgcgggctgctatgaattaccttcaggtgaggtggtgttcgatctgaccgtggccgacggaaacgttttcttctggttcccgccagatgaaaatgtcacaccacccgacgggtttgccaaaaggaacagactcactagtcctacggtacgctgggtatttgatccgaaggcgaaaaagtcagccattagaacgcctggagctggtgatgctgatgtctgggtggctgatgaaagggtcaaaccggcattaacctggctaactaacggcgaattcagccgtatcgatgatcgctttgtaaccaaaccatatcggcacttctggcaggccgtggtagatccatcccggccctacgatttcgagaagtgtgggcctcctgctggggggctgttcaactgtctggggcattatacctggtcagaggaacactatcatgctgggggatcggttcaaaatggtgctgccgagcagcgcgatctgaaagggaagttcggtctggaagacgtgtattttgcggggccaacaatgacttttcaggagccaacattcattccacgtgaaggaggggcagaaggtgagggctatttgatagccttactcaaccatctcgatgagttacggaacgatgtagttatcttcgacgctcagcatctagcgaaaggtccgctggcggttatacatctgccgctaaagctgaagctgggacttcatggcaactgggtagatcaccgtgatatagatgcttggaaacaaaggcgagcagaagggggtgatgtcgggccactcaaagtggcaaccgaacccctaccctggcaaaagaagttagcccagcaaaacggcacgaacggtacacgggcataa

SEQ ID NO: 6 - protein, 595 aa, Thermothielavioides terrestris
  REGION 1..595: note = TtAdo2 amino acid sequence
MAHIHELAAEISNYANNRLTDPSKVRFPRTPVFASMNKPSRFEGDVFDLEISGTIPADIDGTFFRVQPDHRFPPLFEDDIHFNGDGSVTAVRISGGHADLKQRYVHTDRYVHETRARRSLFGRYRNPWTDNESVKGVIRTASNTNVVFWRGVLLALKEDGPPFAMDPVTLETLGRYDFEGQILSPTFTAHPKFDPDTGEMVCFAYEAGGDGSDCSVDVAVWTIDRDGKKTEECWYKAPFAGMIHDCGISKNWLVLALTPIKMDLERMKRGGNKFAWDPNEDQWYAVVPRRGGKSEDITWFRADNGFHGHVAGCYELPSGEVVFDLTVADGNVFFWFPPDENVTPPDGFAKRNRLTSPTVRWVFDPKAKKSAIRTPGAGDADVWVADERVKPALTWLTNGEFSRIDDRFVTKPYRHFWQAVVDPSRPYDFEKCGPPAGGLFNCLGHYTWSEEHYHAGGSVQNGAAEQRDLKGKFGLEDVYFAGPTMTFQEPTFIPREGGAEGEGYLIALLNHLDELRNDVVIFDAQHLAKGPLAVIHLPLKLKLGLHGNWVDHRDIDAWKQRRAEGGDVGPLKVATEPLPWQKKLAQQNGTNGTRA

SEQ ID NO: 7 - DNA, 1683 bp, Penicillium simplicissimum
  source 1..1683: mol_type = unassigned DNA
  misc_feature 1..1683: note = PsVAO nucleotide sequence
atgtccaagacacaggaattcaggcctttgacactgccacccaagctgtcgttaagtgacttcaatgaattcatccaggatattattcgaatcgttggctctgaaaatgttgaagtcattagctcgaaggaccagattgttgacggttcttatatgaaacctacgcacacgcacgatccccatcatgtcatggaccaggactacttccttgcctcagcaattgttgctcctcgcaatgtcgccgatgtgcagtcgattgtcggacttgccaataagttctcatttcccctctggcccatctctattggaagaaattccggatatggcggtgctgcgccacgggttagtggcagtgtcgtgctggacatgggaaagaatatgaacagagttctagaagtgaacgtggaaggcgcatattgcgtggtggagcccggtgtaacttaccacgacttgcataattaccttgaggcgaacaatcttcgagacaaattatggcttgatgtaccggatcttggtggcggttctgttctcggcaatgccgttgagagaggtgtgggctatacgccttacggagatcattggatgatgcacagtgggatggaagtcgtccttgcgaatggcgagcttcttaggactggcatgggggctctacctgatcctaaacgtcccgaaacgatggggctaaagccagaagaccagccatggagcaaaatcgctcatctgtttccttatggcttcggtccctatatagatgggctattcagccaatcgaatatgggaattgttaccaagatcgggatctggttaatgcccaatccagggggttatcaatcctacttgatcacactacccaaagatggtgatttaaaacaagccgtcgatattattcgtccccttcgtctaggcatggcccttcaaaatgttcccactattcgccacattcttttggatgcagcggtgctcggtgacaagcgatcttattcatccaagaccgaacccctctccgacgaggaattagacaagatcgcgaaacagctcaacttgggacgatggaacttttacggggcgctctatggacctgagccgattcgaagggttctctgggaaacgattaaagacgcattctcggcgatcccaggcgtcaagttttattttccggaggacactcctgaaaactccgttctccgcgtgcgtgataagactatgcaaggcattccaacttacgacgagctaaagtggatcgattggctccctaatggtgcgcatctgttcttctctcctattgcgaaggtatctggtgaagatgcaatgatgcaatacgcagtcaccaagaaaaggtgtcaggaggctgggttagattttatcggcactttcacagtcggtatgagagagatgcatcatatcgtttgtattgtgttcaacaagaaggacctaatacaaaagagaaaagtacagtggctgatgagaacccttattgatgactgtgctgcaaatggatggggcgaatatcgaacccatctggccttcatggaccaaattatggaaacctacaactggaacaacagcagcttcctaaggttcaatgaggtcctcaagaatgcggtggatcctaatggcatcattgccccgggaaagtctggtgtttggccgagtcaatacagtcatgttacttggaaactgtaa

SEQ ID NO: 8 - protein, 560 aa, Penicillium simplicissimum
  REGION 1..560: note = PsVAO amino acid sequence
MSKTQEFRPLTLPPKLSLSDFNEFIQDIIRIVGSENVEVISSKDQIVDGSYMKPTHTHDPHHVMDQDYFLASAIVAPRNVADVQSIVGLANKFSFPLWPISIGRNSGYGGAAPRVSGSVVLDMGKNMNRVLEVNVEGAYCVVEPGVTYHDLHNYLEANNLRDKLWLDVPDLGGGSVLGNAVERGVGYTPYGDHWMMHSGMEVVLANGELLRTGMGALPDPKRPETMGLKPEDQPWSKIAHLFPYGFGPYIDGLFSQSNMGIVTKIGIWLMPNPGGYQSYLITLPKDGDLKQAVDIIRPLRLGMALQNVPTIRHILLDAAVLGDKRSYSSKTEPLSDEELDKIAKQLNLGRWNFYGALYGPEPIRRVLWETIKDAFSAIPGVKFYFPEDTPENSVLRVRDKTMQGIPTYDELKWIDWLPNGAHLFFSPIAKVSGEDAMMQYAVTKKRCQEAGLDFIGTFTVGMREMHHIVCIVFNKKDLIQKRKVQWLMRTLIDDCAANGWGEYRTHLAFMDQIMETYNWNNSSFLRFNEVLKNAVDPNGIIAPGKSGVWPSQYSHVTWKL